European Patent Application EP 4 628 070 A1, published October 8, 2025. Title: GOLD NANOZYME COMPRISING GLYCOL CHITOSAN AND GOLD PARTICLES, AND PHARMACEUTICAL COMPOSITION FOR PREVENTING OR TREATING INFLAMMATORY BOWEL DISEASE COMPRISING SAME. Applicant: IUCF-HYU (INDUSTRY-UNIVERSITY COOPERATION FOUNDATION HANYANG UNIVERSITY). Application KR PCT/KR2023/019142, filed November 24, 2023. The sequence listing filed with the application follows.

SEQUENCE LISTING (12 sequences)

SEQ ID NO: 1 - DNA, 20 bp, artificial sequence
  source 1..20: mol_type = other DNA
caggaggcattgctgatgat

SEQ ID NO: 2 - DNA, 18 bp, artificial sequence
  source 1..18: mol_type = other DNA
gaaggctggggctcattt

SEQ ID NO: 3 - DNA, 23 bp, artificial sequence
  source 1..23: mol_type = other DNA
ccctcacactcagatcatcttct

SEQ ID NO: 4 - DNA, 19 bp, artificial sequence
  source 1..19: mol_type = other DNA
gctacgacgtgggctacag

SEQ ID NO: 5 - DNA, 23 bp, artificial sequence
  source 1..23: mol_type = other DNA
tagtccttcctaccccaatttcc

SEQ ID NO: 6 - DNA, 21 bp, artificial sequence
  source 1..21: mol_type = other DNA
ttggtccttagccactccttc

SEQ ID NO: 7 - DNA, 22 bp, artificial sequence
  source 1..22: mol_type = other DNA
gcaactgttcctgaactcaact

SEQ ID NO: 8 - DNA, 21 bp, artificial sequence
  source 1..21: mol_type = other DNA
atcttttggggtccgtcaact

SEQ ID NO: 9 - DNA, 21 bp, artificial sequence
  source 1..21: mol_type = other DNA
ttaaaaacctggatcggaacc

SEQ ID NO: 10 - DNA, 23 bp, artificial sequence
  source 1..23: mol_type = other DNA
gcattagcttcagatttacgggt

SEQ ID NO: 11 - DNA, 20 bp, artificial sequence
  source 1..20: mol_type = other DNA
ccccgctactactccatcag

SEQ ID NO: 12 - DNA, 20 bp, artificial sequence
  source 1..20: mol_type = other DNA
ccactgacacttcgcacaaa